European Patent Application EP 4 198 125 A2, published June 21, 2023. Title: PIF1-LIKE HELICASE AND USE THEREOF. Applicant: Qitan Technology Ltd., Beijing. The sequence listing filed with the application follows.

SEQUENCE LISTING (35 sequences)

SEQ ID NO: 1 - protein, 444 aa, Artificial Sequence
MSLVFEDLKQGQREAFNRIIEVVKKRSGGRITLNGPAGCGKTTLTKFIIDHLVRNGILGVVLAAPTHQAKKVLSKLSGVEANTIHRILKINPNTYEDQDIFEQREMPDLSKCNVLICDEASMYGDKLFGIILRSVPSWCVIIGIGDREQLPPVEPGSDGQTLISPFFTHPSFEQLYLTEVVRSNTPIIDVATEIRMGSWLRENIVDGHGVHEFNSSTALKDYMTEYFNVVKDADDLIETRMLAFTNKSVDKLNSIIRRRLYETETSFIKDEIIVMQEPMIKELEFDGKKFSETIFNNGQLVRIKDAMLTSGFLSARNVSTRQMINYWSLEVETAEDDEEYRVDVIKFLPADQVEKFNYFLAKTATTYREMKNAGKKAPWEDFWKAKRTFLKVRALPVSTIHKAQGVSVNRSFLYTPCIHIAEAQLAKQLAYVGVTRARHDVYYV

SEQ ID NO: 2 - protein, 442 aa, Artificial Sequence
MTDLQFDDLTEGQQNAFNAALEAMKTKGQHITINGPAGTGKTTLTKFLINHLIRTGESGIMLAAPTHQAKKVLSKLAGMEAQTIHSLLKINPTTYEDATLFEQSDVPDLSECRVLICDEVSMYDRELFRILMASVPYWCTIIGLGDIAQIRPVAPNSNIPEVSAFFLNEKFEQVALTEVMRSNAPIIEVATEIRHGKWIRECLLNGEGVHDMVLPTGGSVANFMYKYFDIVKTPEDLFENRMLAFTNKSVGNLNKIIRRKLYQTEVPFINDEVLVMQEPLMRTHKFEGKSFTDVRFNNGELVRVLSCQPITKRLAIRGIDQEDVVKCWHLELRAIETDVVDSICVIEDERQMKIFQHYLSAVAYEFKNSNTGKRPNWSGWWDLRKEFHKVKALPCGTIHKSQGTSVDNVFLYTPCIHSADADLAQQLLYVGATRARNNVYFV

SEQ ID NO: 3 - protein, 453 aa, Artificial Sequence
MSEAESLLAKIVLTDCQKNAIGMVLSDKSHITISGPAGSGKSFLTKILIKKLLELNNGSVVACAPTHQAKIVLSKMSGMTAATIHSILKIHPDTYEDVREFKQSKSDKAKEDLKEVRYLLVDEGSMVDNDLFEILLKSVHPYCQIIAIGDKHQIQPVRHAPGEISPFFTDKRFRLAELKTIVRQQAGNPIIQVATKIRNGGWFETNWDKESGTGVLDVKSVANLMKIYLSKVKTPDDLLNYRMLAYTNDVVNRFNKAIRKQVYNTTEPFVDNEYLVMQEPVMKESEIGGETFTETLLNNGETVKIKEGSIKRQMKYISLPYVDPIQIEIATMTVIRNEVDLTEIDGDLEVELSVVWDADGQVQLDEALSYAASQYKQMGSGKATSRLWESFWQVKGMFTNTKSLGASTFHKSQGTTVIGVCVYTGDMNFAQFEIQTQLGYVGCTRAQKWVMYC

SEQ ID NO: 4 - protein, 454 aa, Artificial Sequence
MSEAASLLAKIILTDCQKTAIDAVLTDKKHITISGPAGSGKSFLTKILIQKLLDLNSGAVITCAPTHQAKIVLSKMSGFTASTIHSVLKIHPDTYEDVREFKQSKSDKAKEDLKAVRYLIVDEASMVDNDLFEILLKSVHPFCQIIAIGDKHQIQPVRHAPGEISPFFTDKRFRLAELKTVVRQQAGNPIIQVATKIRNGGWFETNWDKATGTGVLDVKTIAKMMQIYLSKVKTPEDLLNYRMLAYTNDVVNSFNRVIRKHVYKTTEPFVDNEYLVMQEPVMREEEIGGETFTETLLNNGETVKIIPGSIKRQLKYISLPYVEPIQIEVATMLVERQETDVTDNVDSDKEVEISVVWDASSQVLLDEALSYAASQYKQMGSGKATSRLWESFWQVKGMFVNTKSLGASTFHKSQGTTVIGVCVYTGDMNFAQFEIQTQLGYVGCTRAQKWVIYC

SEQ ID NO: 5 - protein, 441 aa, Artificial Sequence
MNFDDLTVGQKEAFEIVIEAIRTKKHHVMINGPAGTGKTTMTKFILEHLVRNGELGIMLAAPTHQAKKVLSKLSGHQAATIHSILKISPTTYEAESIFEQKEMPDLAKCRVLLCDEGSMYDGALFKILMNTIPSHCTVIGIGDEEQLRPVSPGDSLPSKSPFFSDHRFKQVTLTEVKRSNGPIIKVATEIRNGGWFRECIEDGHGFHGFNGDKPLQQYMMKYFDVVKSPEDLFETRMLAYTNKSVDKLNGIIRRKLYETESPFIVGEVLVMQEPYMKSLEFDGKKFNEIIFNNGQMVRILDCKLTSTFLKARDVSVKQMISYWHLEVETVDEDDDYQRETIKVLADDNEKQKFDMFLAKVATSYRELKSAGRRPHWADFWDAKRTFLKVKALPCSTIHKSQGISVDNAFIYTPCITLADIDLAKQLAYVSSTRARHDVYFV

SEQ ID NO: 6 - protein, 446 aa, Artificial Sequence
MSQEVTFESLNKGQREAFDIITSAIQRRNGERLTLNGPAGTGKTTLTKFIIQHIVRNGVLGVVLAAPTHQAKKVLAKMSGMEANTIHRVLKINPMTYEDQDVFEQREMPDMSKCNVLVCDEASMLDGKIFKIILNSIPPWAVLIGIGDREQIQPVEPGSDGTPQISPFFTHPSFKQVHLTEVMRSNAPIIDVATDIRTGGWLRHHIIDGHGVHEFASTTALKDFMMQYFDVVKTPEDLFETRMLAFTNKSVEKLNNIIRRKLYETEVPFINEEVIVMQEPFIKELEFDGKKFSEIVFNNGEMVRIKDCMLTSMPLIARNVSTKQHINYWALEVETIDPDEEYKIEVIKVLPLDQYQKMDMFLAKVATTYREMKAAGKRPPWDDFWKIKRTFLKVRALPVSTIHKSQGISVNNSFIYTPCIHVAEVQLARQLAYVGLTRARHDAYYV

SEQ ID NO: 7 - protein, 452 aa, Artificial Sequence
MNDLKLEDLNEGQRAAFDAVIKVISTKSMMATTSSCEVKPHITINGPAGTGKTTLTRFLINHLISSGEKGVMLAAPTHQAKKVLAKLSGMEASTIHSLLKINPTTYEDSTVFQQSDDPDLSDCRVLICDEVSMYDRELFRILMASIPPWATIIGLGDIAQIRPVAPNSTTPELSAFFFNDKFQQVSLTEVMRSNAPIIEVATEIRKGGWIRENLVDGQGVHSMVRSNGGSVAAFLTKYFEIVKDPDDLFDNRMLAFTNKSVNDLNNIIRKKLYQTTVPYIKDEVLVMQEPLMRSHTFEGKTFTEVIFNNGELVRIINCREKYVNLFIKGFKGSDSIKVWELEIRGVDSDAVDMIKVIHDEQELNKFQYFMSKSASEFKNARDKRPNWKGWWDLKAQFHKVKPLPCGTIHKSQGSTLDNVFLFTPCIHRADPALAQQLLYVGATRAKHNVYFV

SEQ ID NO: 8 - protein, 454 aa, Artificial Sequence
MVITFDDLTEGQKLAFNEVVDAIKTQNLNLRADTKTHITINGEAGTGKTTLTKFLIDYIIKEGINGVILAAPTHAAKTVLSKLSGMEAETIHSVLKISPTNYEEQTVFEQREIPNLAECRILICDEGSMYDRKLVQLILNTVPKWALVIVLGDKEQIRPVSPGETLPGISPFFTHKKFKQIKLTEVKRSNGPIITVAREILKGQWLRECLDEDGQGVHAYDPESDIPSLHWFLKEYFKVVKTKEDFVNTRVMAYTNKVVNTLNKIIRKRIFNTDEPFIEDEIIVMQGPLTESLIVDGKKVKKLIYNNGQRVRIVRVNKTVHTLRARFVESTKEIDVWTLTVETADKNIDEYHLKDLHIVDEGSELVLKEFLSETANTYRYWELPGKAPWGEFWTIKERYSNVKAEPCSTIHKAQGISVDNAFLCTSGLSSMDPDLVKELIYVGSTRPKHNLYWI

SEQ ID NO: 9 - protein, 441 aa, Artificial Sequence
MKFEDLTVGQKSAFDVVIEAIKTKKFHVMINGPAGTGKTTMTKFILEHLVRNGELGIMLAAPTHQAKKVLSKLSGHEAATIHSVLKISPTTYEAESIFEQKEMPDLAKCRVLFCDEGSMYDGALFKILMNTIPSHCTVIGIGDEEQLRPVSPGDSLPSKSPFFSDSRFKQVTLTEVKRSNGPIIKVATEIRTGGWFRECIEDGHGFHGFGGDKPLQQYMMKYFDVVKSPEDLFETRMLAYTNKSVDKLNGIIRRKLYETENPFIVGEVLVMQEPYMKQLEFDGKKFNEIIFNNGQMIRILDCKLTSTFLKARDVSVKQMISYWHLEVETVDEDDDYQRETIKVLADANEKQKFDMFLAKVATTYRELKSAGRRPHWADFWDAKRTFLKVKALPCSTIHKSQGISVDNTFIYTPCITLADIDLAKQLAYVSATRARHDVYFV

SEQ ID NO: 10 - protein, 443 aa, Artificial Sequence
MTIGFDDLTEGQKCAFETAVELVNSKRKHMTLNGPAGSGKTTWTRFFIDHLVRSGESGVILAAPTHQAKKVLSKLSGVEASTIHSILKINPTTYEENVLFEQKEIPDLAKCRVLICDEASMYDRKLFDILMNSIPSWCIVIALGDKDQLRPVELNSEGKGQISAFFYDPRFEQVFLSEIKRSNSPIIEVATSIRTGGWLYHNLGDDGTGVHGYMNKGSALKDFFGQYFDTVRKPEDLFENRMCAYTNESVNKLNSIIRRKIYDTEDPFVVNEVLVMQEPLTKEIKFEGKRFSEMIFHNGQMVRVVKAEKTSKFLRAKGVSGEQMIRYWSLVVETNDAEDEYFREQICVLSDENEINKYYYFLAKVADAYKSGAVKAHWADFWAAKRAFIKVKALPCSTIHKVQGISVDNCFLYTPCIHKADADLAKQLTYVGATRPRFNLHYV

SEQ ID NO: 11 - protein, 441 aa, Artificial Sequence
MITIDQLTEGQFDSLQRAKVLIQEATKNDGNWNHRTKHLTINGPAGTGKTTMMKFLVSWLRDEGITGVALAAPTHAAKKVLANAVGEEVSTIHSILKINPTTYEEKQFFEQSAPPDLSKIRILICEECSFYDIKLFEILMNSIQPWTIIIGIGDRAQLRPADDKGISRFFTDQRFEQTYLTEIKRSNMPIIEVATEIRNGGWIRENIIDDLGVKQDKSVSEFMTNYFKVVKSIDDLYETRMYAYTNNSVDTLNKIIRKKLYETEQDFIVGEPIVMQEPLIRDINYEGKRFQEIVFNNGEYLEVSEIKPMESVLKCRNIDYQLVLHYYQLKVKSIDTGESGLINTISDKNELNKFYMFLGKVAQDYKSGTIKAFWDDFWKIKNNYHRVKPLPVSTIHKGQGSTVDNSFLYTPCITKYAEPDLASQLLYVGVTRARHNVNFVG

SEQ ID NO: 12 - protein, 185 aa, Artificial Sequence
MGLDNELSLVDGQDRTLTVQQWDTFLNGVFPLDRNRLTREWFHSGRAKYIVAGPGADEFEGTLELGYQIGFPWSLGVGINFSYTTPNILINNGNITAPPFGLNSVITPNLFPGVSISARLGNGPGIQEVATFSVRVSGAKGGVAVSNAHGTVTGAAGGVLLRPFARLIASTGDSVTTYGEPWNMN

SEQ ID NO: 13 - DNA, 7 bp, Artificial Sequence
ttttttt

SEQ ID NO: 14 - DNA, 16 bp, Artificial Sequence
ccgttctcattggtgc

SEQ ID NO: 15 - DNA, 20 bp, Artificial Sequence
tcactatcgcattctcatga

SEQ ID NO: 16 - DNA, 20 bp, Artificial Sequence
tcatgagaatgcgatagtga

SEQ ID NO: 17 - DNA, 10563 bp, Artificial Sequence
atcctgagaccccttttttttgttttgccttttagaattttattcgccattcaggctgcgcaactgttgggaagggcgatcggtgcgggcctcttcgctattacgccagctggcgaaagggggatgtgctgcaaggcgattaagttgggtaacgccagggtttacccagtcacgacgttgtaaaacgacggccagtgaattcgagctcggtacctcgcgaatgcatctagatatcggatcctttttagaatttttacctgggcagacaggactgcgcgggcattcaaatccatgtgggatgcggtgctggatattggtcgtcctgataccgcgcaggagatgctgattaaggcagaggctgcgtataagaaagcagacgacatctggaatctgcgcaaggatgattattttgttaacgatgaagcgcgggcgcgttactgggatgatcgtgaaaaggcccgtcttgcgcttgaagccgcccgaaagaaggctgagcagcagactcaacaggacaaaaatgcgcagcagcagagcgataccgaagcgtcacggctgaaatataccgaagaggcgcagaaggcttacgaacggctgcagacgccgctggagaaatataccgcccgtcaggaagaactgaacaaggcactgaaagacgggaaaatcctgcaggcggattacaacacgctgatggcggcggcgaaaaaggattatgaagcgacgctgaaaaagccgaaacagtccagcgtgaaggtgtctgcgggcgatcgtcaggaagacagtgctcatgctgccctgctgacgcttcaggcagaactccggacgctggagaagcatgccggagcaaatgagaaaatcagccagcagcgccgggatttgtggaaggcggagagtcagttcgcggtactggaggaggcggcgcaacgtcgccagctgtctgcacaggagaaatccctgctggcgcataaagatgagacgctggagtacaaacgccagctggctgcacttggcgacaaggttacgtatcaggagcgcctgaacgcgctggcgcagcaggcggataaattcgcacagcagcaacgggcaaaacgggccgccattgatgcgaaaagccgggggctgactgaccggcaggcagaacgggaagccacggaacagcgcctgaaggaacagtatggcgataatccgctggcgctgaataacgtcatgtcagagcagaaaaagacctgggcggctgaagaccagcttcgcgggaactggatggcaggcctgaagtccggctggagtgagtgggaagagagcgccacggacagtatgtcgcaggtaaaaagtgcagccacgcagacctttgatggtattgcacagaatatggcggcgatgctgaccggcagtgagcagaactggcgcagcttcacccgttccgtgctgtccatgatgacagaaattctgcttaagcaggcaatggtggggattgtcgggagtatcggcagcgccattggcggggctgttggtggcggcgcatccgcgtcaggcggtacagccattcaggccgctgcggcgaaattccattttgcaaccggaggatttacgggaaccggcggcaaatatgagccagcggggattgttcaccgtggtgagtttgtcttcacgaaggaggcaaccagccggattggcgtggggaatctttaccggctgatgcgcggctatgccaccggcggttatgtcggtacaccgggcagcatggcagacagccggtcgcaggcgtccgggacgtttgagcagaataaccatgtggtgattaacaacgacggcacgaacgggcagataggtccggctgctctgaaggcggtgtatgacatggcccgcaagggtgcccgtgatgaaattcagacacagatgcgtgatggtggcctgttctccggaggtggacgatgaagaccttccgctggaaagtgaaacccggtatggatgtggcttcggtcccttctgtaagaaaggtgcgctttggtgatggctattctcagcgagcgcctgccgggctgaatgccaacctgaaaacgtacagcgtgacgctttctgtcccccgtgaggaggccacggtactggagtcgtttctggaagagcacgggggctggaaatcctttctgtggacgccgccttatgagtggcggcagataaaggtgacctgcgcaaaatggtcgtcgcgggtcagtatgctgcgtgttgagttcagcgcagagtttgaacaggtggtgaactgatgcaggatatccggcaggaaacactgaatgaatgcacccgtgcggagcagtcggccagcgtggtgctctgggaaatcgacctgacagaggtcggtggagaacgttattttttctgtaatgagcagaacgaaaaaggtgagccggtcacctggcaggggcgacagtatcagccgtatcccattcaggggagcggttttgaactgaatggcaaaggcaccagtacgcgccccacgctgacggtttctaacctgtacggtatggtcaccgggatggcggaagatatgcagagtctggtcggcggaacggtggtccggcgtaaggtttacgcccgttttctggatgcggtgaacttcgtcaacggaaacagttacgccgatccggagcaggaggtgatcagccgctggcgcattgagcagtgcagcgaactgagcgcggtgagtgcctcctttgtactgtccacgccgacggaaacggatggcgctgtttttccgggacgtatcatgctggccaacacctgcacctggacctatcgcggtgacgagtgcggttatagcggtccggctgtcgcggatgaatatgaccagccaacgtccgatatcacgaaggataaatgcagcaaatgcctgagcggttgtaagttccgcaataacgtcggcaactttggcggcttcctttccattaacaaactttcgcagtaaatcccatgacacagacagaatcagcgattctggcgcacgcccggcgatgtgcgccagcggagtcgtgcggcttcgtggtaagcacgccggagggggaaagatatttcccctgcgtgaatatctccggtgagccggaggctatttccgtatgtcgccggaagactggctgcaggcagaaatgcagggtgagattgtggcgctggtccacagccaccccggtggtctgccctggctgagtgaggccgaccggcggctgcaggtgcagagtgatttgccgtggtggctggtctgccgggggacgattcataagttccgctgtgtgccgcatctcaccgggcggcgctttgagcacggtgtgacggactgttacacactgttccgggatgcttatcatctggcggggattgagatgccggactttcatcgtgaggatgactggtggcgtaacggccagaatctctatctggataatctggaggcgacggggctgtatcaggtgccgttgtcagcggcacagccgggcgatgtgctgctgtgctgttttggttcatcagtgccgaatcacgccgcaatttactgcggcgacggcgagctgctgcaccatattcctgaacaactgagcaaacgagagaggtacaccgacaaatggcagcgacgcacacactccctctggcgtcaccgggcatggcgcgcatctgcctttacggggatttacaacgatttggtcgccgcatcgaccttcgtgtgaaaacgggggctgaagccatccgggcactggccacacagctcccggcgtttcgtcagaaactgagcgacggctggtatcaggtacggattgccgggcgggacgtcagcacgtccgggttaacggcgcagttacatgagactctgcctgatggcgctgtaattcatattgttcccagagtcgccggggccaagtcaggtggcgtattccagattgtcctgggggctgccgccattgccggatcattctttaccgccggagccacccttgcagcatggggggcagccattggggccggtggtatgaccggcatcctgttttctctcggtgccagtatggtgctcggtggtgtggcgcagatgctggcaccgaaagccagaactccccgtatacagacaacggataacggtaagcagaacacctatttctcctcactggataacatggttgcccagggcaatgttctgcctgttctgtacggggaaatgcgcgtggggtcacgcgtggtttctcaggagatcagcacggcagacgaaggggacggtggtcaggttgtggtgattggtcgctgatgcaaaatgttttatgtgaaaccgcctgcgggcggttttgtcatttatggagcgtgaggaatgggtaaaggaagcagtaaggggcataccccgcgcgaagcgaaggacaacctgaagtccacgcagttgctgagtgtgatcgatgccatcagcgaagggccgattgaaggtccggtggatggcttaaaaagcgtgctgctgaacagtacgccggtgctggacactgaggggaataccaacatatccggtgtcacggtggtgttccgggctggtgagcaggagcagactccgccggagggatttgaatcctccggctccgagacggtgctgggtacggaagtgaaatatgacacgccgatcacccgcaccattacgtctgcaaacatcgaccgtctgcgctttaccttcggtgtacaggcactggtggaaaccacctcaaagggtgacaggaatccgtcggaagtccgcctgctggttcagatacaacgtaacggtggctgggtgacggaaaaagacatcaccattaagggcaaaaccacctcgcagtatctggcctcggtggtgatgggtaacctgccgccgcgcccgtttaatatccggatgcgcaggatgacgccggacagcaccacagaccagctgcagaacaaaacgctctggtcgtcatacactgaaatcatcgatgtgaaacagtgctacccgaacacggcactggtcggcgtgcaggtggactcggagcagttcggcagccagcaggtgagccgtaattatcatctgcgcgggcgtattctgcaggtgccgtcgaactataacccgcagacgcggcaatacagcggtatctgggacggaacgtttaaaccggcatacagcaacaacatggcctggtgtctgtgggatatgctgacccatccgcgctacggcatggggaaacgtcttggtgcggcggatgtggataaatgggcgctgtatgtcatcggccagtactgcgaccagtcagtgccggacggctttggcggcacggagccgcgcatcacctgtaatgcgtacctgaccacacagcgtaaggcgtgggatgtgctcagcgatttctgctcggcgatgcgctgtatgccggtatggaacgggcagacgctgacgttcgtgcaggaccgaccgtcggataagacgtggacctataaccgcagtaatgtggtgatgccggatgatggcgcgccgttccgctacagcttcagcgccctgaaggaccgccataatgccgttgaggtgaactggattgacccgaacaacggctgggagacggcgacagagcttgttgaagatacgcaggccattgcccgttacggtcgtaatgttacgaagatggatgcctttggctgtaccagccgggggcaggcacaccgcgccgggctgtggctgattaaaacagaactgctggaaacgcagaccgtggatttcagcgtcggcgcagaagggcttcgccatgtaccgggcgatgttattgaaatctgcgatgatgactatgccggtatcagcaccggtggtcgtgtgctggcggtgaacagccagacccggacgctgacgctcgaccgtgaaatcacgctgccatcctccggtaccgcgctgataagcctggttgacggaagtggcaatccggtcagcgtggaggttcagtccgtcaccgacggcgtgaaggtaaaagtgagccgtgttcctgacggtgttgctgaatacagcgtatgggagctgaagctgccgacgctgcgccagcgactgttccgctgcgtgagtatccgtgagaacgacgacggcacgtatgccatcaccgccgtgcagcatgtgccggaaaaagaggccatcgtggataacggggcgcactttgacggcgaacagagtggcacggtgaatggtgtcacgccgccagcggtgcagcacctgaccgcagaagtcactgcagacagcggggaatatcaggtgctggcgcgatgggacacaccgaaggtggtgaagggcgtgagtttcctgctccgtctgaccgtaacagcggacgacggcagtgagcggctggtcagcacggcccggacgacggaaaccacataccgcttcacgcaactggcgctggggaactacaggctgacagtccgggcggtaaatgcgtgggggcagcagggcgatccggcgtcggtatcgttccggattgccgcaccggcagcaccgtcgaggattgagctgacgccgggctattttcagataaccgccacgccgcatcttgccgtttatgacccgacggtacagtttgagttctggttctcggaaaagcagattgcggatatcagacaggttgaaaccagcacgcgttatcttggtacggcgctgtactggatagccgccagtatcaatatcaaaccgggccatgattattacttttatatccgcagtgtgaacaccgttggcaaatcggcattcgtggaggccgtcggtcgggcgagcgatgatgcggaaggttacctggattttttcaaaggcaagataaccgaatcccatctcggcaaggagctgctggaaaaagtcgagctgacggaggataacgccagcagactggaggagttttcgaaagagtggaaggatgccagtgataagtggaatgccatgtgggctgtcaaaattgagcagaccaaagacggcaaacattatgtcgcgggtattggcctcagcatggaggacacggaggaaggcaaactgagccagtttctggttgccgccaatcgtatcgcatttattgacccggcaaacgggaatgaaacgccgatgtttgtggcgcagggcaaccagatattcatgaacgacgtgttcctgaagcgcctgacggcccccaccattaccagcggcggcaatcctccggccttttccctgacaccggacggaaagctgaccgctaaaaatgcggatatcagtggcagtgtgaatgcgaactccgggacgctcagtaatgtgacgatagctgaaaactgtacgataaacggtacgctgagggcggaaaaaatcgtcggggacattgtaaaggcggcgagcgcggcttttccgcgccagcgtgaaagcagtgtggactggccgtcaggtacccgtactgtcaccgtgaccgatgaccatccttttgatcgccagatagtggtgcttccgctgacgtttcgcggaagtaagcgtactgtcagcggcaggacaacgtattcgatgtgttatctgaaagtactgatgaacggtgcggtgatttatgatggcgcggcgaacgaggcggtacaggtgttctcccgtattgttgacatgccagcgggtcggggaaacgtgatcctgacgttcacgcttacgtccacacggcattcggcagatattccgccgtatacgtttgccagcgatgtgcaggttatggtgattaagaaacaggcgctgggcatcagcgtggtctgagtgtgttacagaggttcgtccgggaacgggcgttttattataaaacagtgagaggtgaacgatgcgtaatgtgtgtattgccgttgctgtctttgccgcacttgcggtgacagtcactccggcccgtgcggaaggtggacatggtacgtttacggtgggctattttcaagtgaaaccgggtacattgccgtcgttgtcgggcggggataccggtgtgagtcatctgaaagggattaacgtgaagtaccgttatgagctgacggacagtgtgggggtgatggcttccctggggttcgccgcgtcgaaaaagagcagcacagtgatttttttctagatttttagaatttttaagcttgcttggcgtaatcatggtcatagctgtttcctgtgtgaaattgttatccgctcacaattccacacaacatacgagccggaagcataaagtgtaaagcctggggtgcctaatgagtgagctaactcacattaattgcgttgcgctcactgcccgctttccagtcgggaaacctgtcgtgccagctgcattaatgaatcggccaacgcgcggggagaggcggtttgcgtattgggcgcactaccgcttcctcgctcactgactcgctgcgctcggtcgttcggctgcggcgagcggtatcagctcactcaaaggcggtaatacggttatccacagaatcaggggataacgcaggaaagaacatgtgagcaaaaggccagcaaaaggccaggaaccgtaaaaaggccgcgttgctggcgtttttccataggctccgcccccctgacgagcatcacaaaaatcgacgctcaagtcagaggtggcgaaacccgacaggactataaagataccaggcgtttccccctggaagctccctcgtgcgctctcctgttccgaccctgccgcttaccggatacctgtccgcctttctcccttcgggaagcgtggcgctttctcatagctcacgctgtaggtatctcagttcggtgtaggtcgttcgctccaagctgggctgtgtgcacgaaccccccgttcagcccgaccgctgcgccttatccggtaactatcgtcttgagtccaacccggtaagacacgacttatcgccactggcagcagccactggtaacaggattagcagagcgaggtatgtaggcggtgctacagagttcttgaagtggtggcctaactacggctacactagaagaacagtatttggtatctgcgctctgctgaagccagttaccttcggaaaaagagttggtagctcttgatccggcaaacaaaccaccgctggtagcggtggtttttttgtttgcaagcagcagattacgcgcagaaaaaaaggatctcaagaagatcctttgatcttttctacggggtctgacgctcagtggaacgaaaactcacgttaagggattttggtcatgagattatcaaaaaggatcttcacctagatccttttaaattaaaaatgaagttttaaatcaatctaaagtatatatgagtaaacttggtctgacagttaccaatgcttaatcagtgaggcacctatctcagcgatctgtctatttcgttcatccatagttgcctgactccccgtcgtgtagataactacgatacgggagggcttaccatctggccccagtgctgcaatgataccgcgtgaaccacgctcaccggctccagatttatcagcaataaaccagccagccggaagggccgagcgcagaagtggtcctgcaactttatccgcctccatccagtctattaattgttgccgggaagctagagtaagtagttcgccagttaatagtttgcgcaacgttgttgccattgctacaggcatcgtggtgtcacgctcgtcgtttggtatggcttcattcagctccggttcccaacgatcaaggcgagttacatgatcccccatgttgtgcaaaaaagcggttagctccttcggtcctccgatcgttgtcagaagtaagttggccgcagtgttatcactcatggttatggcagcactgcataattctcttactgtcatgccatccgtaagatgcttttctgtgactggtgagtactcaaccaagtcattctgagaatagtgtatgcggcgaccgagttgctcttgcccggcgtcaatacgggataataccgcgccacatagcagaactttaaaagtgctcatcattggaaaacgttcttcggggcgaaaactctcaaggatcttaccgctgttgagatccagttcgatgtaacccactcgtgcacccaactgatcttcagcatcttttactttcaccagcgtttctgggtgagcaaaaacaggaaggcaaaatgccgcaaaaaagggaataagggcgacacggaaatgttgaatactcatactcttcctttttcaatattattgaagcatttatcagggttattgtctcatgagcggatacatatttgaatgtatttagaaaaataaacaaataggggttccgcgcacatttccccgaaaagtgccacctgacgtctaagaaaccattattatcatgacattaacctataaaaataggcgtatcacgaggccctttcgtctcgcgcgtttcggtgatgacggtgaaaacctctgacacatgcagctcccggagacggtcacagcttgtctgtaagcggatgccgggagcagacaagcccgtcagggcgcgtcagcgggtgttggcgggtgtcggggctggcttaactatgcggcatcagagcagattgtactgagagtgcaccatatgcggtgtgaaataccgcacaggtctctaagctctgtctcttatacacatct

SEQ ID NO: 18 - DNA, 83 bp, Artificial Sequence
tttttttttttttttttttttttttttttttttttttttttttttttttttcgctgctccacaggtctcagcttgagcagcga

SEQ ID NO: 19 - DNA, 33 bp, Artificial Sequence
tcgctgctcaagctgagacctgtggagcagcga

SEQ ID NO: 20 - DNA, 90 bp, Artificial Sequence
ttttttttttttttttttttttttttttttttttttttttttttttttttacagaatagggctaacaaacaagaaacataaacagaatag

SEQ ID NO: 21 - DNA, 40 bp, Artificial Sequence
ctattctgtttatgtttcttgtttgttagccctattctgt

SEQ ID NO: 22 - DNA, 40 bp, Artificial Sequence
acagaatagggctaacaaacaagaaacataaacagaatag

SEQ ID NO: 23 - DNA, 90 bp, Artificial Sequence
ctattctgtttatgtttcttgtttgttagccctattctgtaaaaaaaaaaaaaaaaaaaaaaaaaaaaaaaaaaaaaaaaaaaaaaaaaa

SEQ ID NO: 24 - DNA, 142 bp, Artificial Sequence
atccttttttttcagagattttttttcagagattttttttcagagattttttttaatgtacttcgttcagttacgtattgctttttttttaatgtacttcgttcagttacgtattgcttttttttttttttttttttttttt

SEQ ID NO: 25 - DNA, 1335 bp, Artificial Sequence
atgtctctggttttcgaagacctgaaacagggtcagcgtgaagcgttcaaccgtatcatcgaagttgttaaaaaacgttctggtggtcgtatcaccctgaacggtccggctggttgcggtaaaaccaccctgaccaaattcatcatcgaccacctggttcgtaacggtatcctgggtgttgttctggctgctccgacccaccaggctaaaaaagttctgtctaaactgtctggtgttgaagctaacaccatccaccgtatcctgaaaatcaacccgaacacctacgaatgccaggacatcttcgaacagcgtgaaatgccggacctgtctaaatgcaacgttctgatctgcgacgaagcttctatgtacggtgacaaactgttcggtatcatcctgcgttctgttccgtcttgggcggttatcatcggtatcggtgaccgtgaacagctgccgccggttgaaccgggttctgacggtcagaccctgatctctccgttcttcacccacccgtctttcgaacagctgtacctgaccgaagttgttcgttctaacaccccgatcatcgacgttgctaccgaaatccgtatgggttcttggctgcgtgaaaacatcgttgacggtcacggtgttcacgaatttaactcttctaccgctctgaaagactacatgaccgaatacttcaacgttgttaaagacgctgacgacctgatcgaaacccgtatgctggctttcaccaacaaatctgttgacaaactgaactctatcatccgtcgtcgtctgtacgaaaccgaaacctctttcatcaaagacgaaatcatcgttatgcaggaaccgatgatcaaagaactggaatttgacggtaaaaaattctctgaaaccatcttcaacaacggtcagctggttcgtatcaaagacgctatgctgacctctggtttcctgtctgctcgtaacgtttctacccgtcagatgatcaactactggtctctggaagttgaaaccgctgaagacgacgaagaataccgtgttgacgttatcaaattcctgccggctgaccaggttgaaaaattcaactacttcctggctaaaacctgcaccacctaccgtgaaatgaaaaacgctggtaaaaaagctccgtgggaagacttctggaaagctaaacgtaccttcctgaaagttcgtgctctgccggtttctaccatccacaaagctcagggtgtttctgttaaccgttctttcctgtacaccccgtgcatccacatcgctgaagctcagctggctaaacagctggcttacgttggtgttacccgtgctcgtcatgacgtatactacgtataa

SEQ ID NO: 26 - DNA, 1329 bp, Artificial Sequence
atgaccgacctgcagtttgacgatctgaccgagggtcagcaaaacgcgttcaacgcggcgctggaagcgatgaagaccaaaggtcaacacatcaccattaacggtccggcgggcaccggcaagaccaccctgaccaaatttctgatcaaccacctgattcgtaccggcgagagcggtatcatgctggcggcgccgacccaccaggcgaagaaagtgctgagcaagctggcgggcatggaagcgcaaaccatccacagcctgctgaaaattaacccgaccacctacgagtgcgcgaccctgtttgaacagagcgacgtgccggatctgagcgagtgccgtgtgctgatctgcgacgaagttagcatgtacgatcgtgaactgttccgtattctgatggcgagcgttccgtattggtgcaccatcattggtctgggcgatatcgcgcagattcgtccggtggcgccgaacagcaacatcccggaagtgagcgcgttctttctgaacgagaagtttgaacaagtggcgctgaccgaagttatgcgtagcaacgcgccgatcattgaggtggcgaccgaaatccgtcacggtaaatggattcgtgagtgcctgctgaacggtgaaggcgtgcacgacatggttctgccgaccggtggcagcgtggcgaacttcatgtacaagtacttcgacatcgttaagaccccggaggacctgttcgaaaaccgtatgctggcgttcaccaacaagagcgtgggcaacctgaacaagatcattcgtcgtaaactgtaccagaccgaggttccgttcattaacgacgaggtgctggttatgcaagaaccgctgatgcgtacccacaagttcgagggcaagagcttcaccgatgttcgtttcaacaacggcgaactggtgcgtgttctgagctgccagccgatcaccaagcgtctggcgatccgtggtattgaccaagaagatgtggttaaatgctggcacctggagctgcgtgcgatcgaaaccgacgtggttgatagcatctgcgtgattgaggatgaacgtcagatgaaaatttttcaacactacctgagcgcggtttgctatgagttcaagaacagcaacaccggtaaacgtccgaactggagcggttggtgggacctgcgtaaggaatttcacaaggtgaaagcgctgccgtgcggcaccatccacaaaagccagggcaccagcgtggataacgttttcctgtataccccgtgcattcacagcgcggacgcggatctggcgcagcaactgctgtacgttggtgcgacccgtgcgcgtaacaacgtgtatttcgtttaa

SEQ ID NO: 27 - DNA, 1362 bp, Artificial Sequence
atgagcgaggcggaaagcctgctggcgaagatcgttctgaccgactgccagaaaaacgcgattggtatggtgctgagcgataagagccacatcaccattagcggtccggcgggtagcggcaagagcttcctgaccaaaatcctgattaagaaactgctggaactgaacaacggtagcgtggttgcgtgcgcgccgacccaccaggcgaagatcgttctgagcaaaatgagcggcatgaccgcggcgaccattcacagcatcctgaagattcacccggacacctacgagtgcgtgcgtgagttcaagcaaagcaaaagcgacaaggcgaaagaggatctgaaagaagttcgttacctgctggttgacgaaggtagcatggttgacaacgacctgttcgagatcctgctgaagagcgtgcacccgtactgccagatcattgcgatcggtgacaaacaccagattcaaccggttcgtcacgcgccgggcgaaattagcccgttctttaccgataagcgtttccgtctggcggagctgaaaaccatcgttcgtcagcaagcgggcaacccgatcattcaggtggcgaccaagattcgtaacggtggctggtttgagaccaactgggacaaagaaagcggcaccggtgtgctggacgttaagagcgtggcgaacctgatgaaaatctatctgagcaaggtgaaaaccccggacgatctgctgaactaccgtatgctggcgtataccaacgacgtggttaaccgtttcaacaaggcgatccgtaaacaggtttacaacaccaccgagccgtttgtggataacgaatatctggttatgcaagagccggtgatgaaagagagcgaaattggtggcgagaccttcaccgaaaccctgctgaacaacggtgaaaccgttaagatcaaagagggcagcattaagcgtcagatgaaatacatcagcctgccgtatgtggacccgatccaaattgaaatcgcgaccatgaccgttatccgtaacgaggtggatctgaccgaaattgacggtgacctggaagtggaactgagcgtggtttgggacgcggatggccaggtgcaactggacgaagcgctgagctactgcgcgagccagtataagcaaatgggtagcggcaaagcgaccagccgtctgtgggagagcttctggcaggttaagggcatgtttaccaacaccaaaagcctgggcgcgagcacctttcacaagagccaaggcaccaccgtgatcggcgtgtgcgtttacaccggtgatatgaacttcgcgcagtttgagattcagacccaactgggttacgttggctgcacccgtgcgcaaaaatgggtgatgtattgctaa

SEQ ID NO: 28 - DNA, 1365 bp, Artificial Sequence
atgagcgaggcggcgagcctgctggcgaaaatcattctgaccgactgccagaagaccgcgatcgacgcggtgctgaccgataagaaacacatcaccattagcggtccggcgggtagcggcaagagcttcctgaccaaaatcctgattcagaagctgctggatctgaacagcggtgcggtgatcacctgcgcgccgacccaccaagcgaaaattgttctgagcaagatgagcggcttcaccgcgagcaccatccacagcgtgctgaaaattcacccggacacctacgaatgcgttcgtgagtttaagcagagcaaaagcgacaaggcgaaagaagatctgaaggcggtgcgttatctgatcgttgacgaggcgagcatggtggacaacgacctgttcgaaattctgctgaaaagcgttcacccgttttgccaaatcattgcgatcggtgacaagcaccagattcagccggtgcgtcatgcgccgggtgaaatcagcccgttctttaccgataaacgtttccgtctggcggaactgaagaccgtggttcgtcagcaagcgggcaacccgatcattcaggttgcgaccaaaattcgtaacggtggctggtttgagaccaactgggacaaggcgaccggcaccggtgtgctggacgttaagaccatcgcgaaaatgatgcaaatttacctgagcaaggtgaaaaccccggaagacctgctgaactaccgtatgctggcgtataccaacgatgtggttaacagcttcaaccgtgtgatccgtaagcacgtttacaaaaccaccgaaccgtttgttgataacgagtatctggtgatgcaggaaccggttatgcgtgaggaagagattggtggcgaaaccttcaccgagaccctgctgaacaacggcgagaccgtgaaaatcattccgggcagcatcaagcgtcaactgaaatacattagcctgccgtatgttgaaccgatccagattgaggtggcgaccatgctggttgaacgtcaagagaccgacgtgaccgataacgttgacagcgataaggaagtggagatcagcgtggtttgggacgcgagcagccaggttctgctggatgaggcgctgagctactgcgcgagccagtataaacaaatgggtagcggcaaggcgaccagccgtctgtgggagagcttctggcaggtgaaaggcatgtttgttaacaccaagagcctgggcgcgagcacctttcacaaaagccaaggcaccaccgttatcggcgtgtgcgtttataccggtgacatgaacttcgcgcagtttgaaattcagacccaactgggttacgtgggctgcacccgtgcgcaaaagtgggttatctattgctaa

SEQ ID NO: 29 - DNA, 1326 bp, Artificial Sequence
atgaacttcgacgacctgaccgttggtcagaaagaagcgttcgaaatcgttatcgaagctatccgtaccaaaaaacaccacgttatgatcaacggtccggctggtaccggtaaaaccaccatgaccaaattcatcctggaacacctggttcgtaacggtgaactgggtatcatgctggctgctccgacccaccaggctaaaaaagttctgtctaaactgtctggtcaccaggctgctaccatccactctatcctgaaaatctctccgaccacctacgaatgcgaatctatcttcgaacagaaagaaatgccggacctggctaaatgccgtgttctgctgtgcgacgaaggttctatgtacgacggtgctctgttcaaaatcctgatgaacaccatcccgtctcacgcgaccgttatcggtatcggtgacgaagaacagctgcgtccggtaagcccgggtgactctctgccgtctaaatctccgttcttctctgaccaccgtttcaaacaggttaccctgaccgaagttaaacgttctaacggtccgatcatcaaagttgctaccgaaatccgtaacggtggttggttccgtgaatgcatcgaagacggtcacggtttccacggtttcaacggtgacaaaccgctgcagcagtacatgatgaaatacttcgacgttgttaaatctccggaagacctgttcgaaacccgtatgctggcttacaccaacaaatctgttgacaaactgaacggtatcatccgtcgtaaactgtacgaaaccgaatctccgttcatcgttggtgaagttctggttatgcaggaaccgtacatgaaatctctggaatttgacggtaaaaaattcaacgaaatcatcttcaacaacggtcagatggttcgtatcctggactgcaaactgacctctaccttcctgaaagctcgtgacgtttctgttaaacagatgatctcttactggcacctggaagttgaaaccgttgacgaagacgacgactaccagcgtgaaaccatcaaagttctggctgacgacaacgaaaaacagaaattcgacatgttcctggctaaagtttgcacctcttaccgtgaactgaaatctgctggtcgtcgtccgcactgggctgacttctgggacgctaaacgtaccttcctgaaagttaaagctctgccgtgctctaccatccacaaatctcagggtatctctgttgacaacgctttcatctacaccccgtgcatcaccctggctgacatcgacctggctaaacagctggcttacgtttcttctacccgtgctcgtcatgacgtgtacttcgtctaa

SEQ ID NO: 30 - DNA, 1341 bp, Artificial Sequence
atgtctcaggaagttaccttcgaatctctgaacaaaggtcagcgtgaagcgttcgacatcatcacctctgctatccagcgtcgtaacggtgaacgtctgaccctgaacggtccggctggtaccggtaaaaccaccctgaccaaattcatcatccagcacatcgttcgtaacggtgttctgggtgttgttctggctgctccgacccaccaggctaaaaaagttctggctaaaatgtctggtatggaagctaacaccatccaccgtgttctgaaaatcaacccgatgacctacgaatgccaggacgttttcgaacagcgtgaaatgccggacatgtctaaatgcaacgttctggtttgcgacgaagcgtccatgctggacggtaaaatcttcaaaatcatcctgaactctatcccgccgtgggcggttctgatcggtatcggtgaccgtgaacagatccagccggttgaaccgggttctgacggtaccccgcagatctctccgttcttcacccacccgtctttcaaacaggttcacctgaccgaagttatgcgttctaacgctccgatcatcgacgttgctaccgacatccgtaccggtggttggctgcgtcaccacatcatcgacggtcacggtgttcacgaatttgcttctaccaccgctctgaaagacttcatgatgcagtatttcgacgttgttaaaaccccggaagacctgttcgaaacccgtatgctggctttcaccaacaaatctgttgaaaaactgaacaacatcatccgtcgtaaactgtacgaaaccgaagttccgttcatcaacgaagaagttatcgttatgcaggaaccgttcatcaaagaactggaatttgacggtaaaaaattctctgaaatcgttttcaacaacggtgaaatggttcgtatcaaagactgcatgctgacctctatgccgctgatcgctcgtaacgtttctaccaaacagcacatcaactactgggctctggaagttgaaaccatcgacccggacgaagaatacaaaatcgaagttatcaaagttctgccgctggaccagtaccagaaaatggacatgttcctggctaaagtttgcaccacctaccgtgaaatgaaagctgctggtaaacgtccgccgtgggacgacttctggaaaatcaaacgtaccttcctgaaagttcgtgctctgccggtttctaccatccacaaatctcagggtatctctgttaacaactctttcatctacaccccgtgcatccacgttgctgaagttcagctggctcgtcagctggcttacgttggtctgacccgtgctcgtcacgacgcttactacgtttaa

SEQ ID NO: 31 - DNA, 1359 bp, Artificial Sequence
atgaacgacctgaaactggaagacctgaacgaaggtcagcgtgctgctttcgacgctgttatcaaagttatctctaccaaatctatgatggctaccacctcttcttgcgaagttaaaccgcacatcaccatcaacggtccggctggtaccggtaaaactactctgacccgtttcctgatcaaccatctgatctcttctggtgaaaaaggtgttatgctggctgctccgacccaccaggctaaaaaagttctggctaaactgtctggtatggaagcgtctaccatccactctctgctgaaaatcaacccgaccacctacgaatgctctaccgttttccagcagtctgacgacccggacctgtctgactgccgtgttctgatctgcgacgaagtttctatgtacgaccgtgaactgttccgtatcctgatggcttctatcccgccgtgggcgaccatcatcggtctgggtgacatcgctcagatccgtccggttgctccgaactctaccaccccggaactgtctgctttcttcttcaacgacaaattccagcaggtttctctgaccgaagttatgcgttctaacgctccgatcatcgaagttgctaccgaaatccgtaaaggtggttggattcgtgaaaacctggttgacggtcagggtgttcactctatggttcgttctaacggtggttctgttgctgctttcctgaccaaatacttcgaaatcgttaaagacccggacgacctgttcgacaaccgtatgctggctttcaccaacaaatctgttaacgacctgaacaacatcatccgtaaaaaactgtaccagaccaccgttccgtacatcaaagacgaagttctggttatgcaggaaccgctgatgcgttctcacaccttcgaaggtaaaaccttcaccgaagttatcttcaacaacggtgaactggttcgtatcatcaactgccgtgaaaaatacgttaacctgttcatcaaaggtttcaaaggttctgactctatcaaagtttgggaactggaaatccgtggtgttgactctgacgctgttgacatgatcaaagttatccacgacgaacaggaactgaacaaattccagtacttcatgtctaaatcttgctctgaatttaaaaacgctcgtgacaaacgtccgaactggaaaggttggtgggacctgaaagctcagttccacaaagttaaaccgctgccgtgcggtaccatccacaaatctcagggttctaccctggacaacgttttcctgttcaccccgtgcatccaccgtgctgacccggctctggctcagcagctgctgtacgttggtgctacccgtgctaaacacaacgtttacttcgtttaa

SEQ ID NO: 32 - DNA, 1365 bp, Artificial Sequence
atggttatcaccttcgacgacctgaccgaaggtcagaaactggctttcaacgaagttgttgacgctatcaaaacccagaacctgaacctgcgtgctgacaccaaaacccacatcaccatcaacggtgaagctggtaccggtaaaaccaccctgaccaaattcctgatcgactacatcatcaaagaaggtatcaacggtgttatcctggctgctccgacccacgctgctaaaaccgttctgtctaaactgtctggtatggaagctgaaaccatccactctgttctgaaaatctctccgaccaactacgaatgccagaccgttttcgaacagcgtgaaatcccgaacctggctgaatgccgtatcctgatctgcgacgaaggttctatgtacgaccgtaaactggttcagctgatcctgaacaccgttccgaaatgggcgctggttatcgttctgggtgacaaagaacagatccgtccggtttctccgggtgaaaccctgccgggtatctctccgttcttcacccacaaaaaattcaaacagatcaaactgaccgaagttaaacgttctaacggtccgatcatcaccgttgctcgtgaaatcctgaaaggtcagtggctgcgtgaatgcctggacgaagacggtcagggtgttcacgcttacgacccggaatctgacatcccgtctctgcactggttcctgaaagaatacttcaaagttgttaaaaccaaagaagacttcgttaacacccgtgttatggcttacaccaacaaagttgttaacaccctgaacaaaatcatccgtaaacgtatcttcaacaccgacgaaccgttcatcgaagacgaaatcatcgttatgcagggtccgctgaccgaatctctgatcgttgacggtaaaaaagttaaaaaactgatctacaacaacggtcagcgtgttcgtatcgttcgtgttaacaaaaccgttcacaccctgcgtgctcgtttcgttgaatctaccaaagaaatcgacgtttggaccctgaccgttgaaaccgctgacaaaaacatcgacgaataccacctgaaagacctgcacatcgttgacgaaggttctgaactggttctgaaagaattcctgtctgaaacctgcaacacctaccgttactgggaactgccgggtaaagctccgtggggtgaattctggaccatcaaagaacgttactctaacgttaaagctgaaccgtgctctaccatccacaaagctcagggtatctctgttgacaacgctttcctgtgcacctctggtctgtcttctatggacccggacctggttaaagaactgatctacgttggttctacccgtccgaaacacaacctgtactggatctaa

SEQ ID NO: 33 - DNA, 1326 bp, Artificial Sequence
atgaaattcgaagacctgaccgttggtcagaaatctgctttcgacgttgttatcgaagctatcaaaaccaaaaaattccacgttatgatcaacggtccggctggtaccggtaaaaccaccatgaccaaattcatcctggaacacctggttcgtaacggtgaactgggtatcatgctggctgctccgacccaccaggctaaaaaagttctgtctaaactgtctggtcacgaagctgctaccatccactctgttctgaaaatctctccgaccacctacgaatgcgaatctatcttcgaacagaaagaaatgccggacctggctaaatgccgtgttctgttctgcgacgaaggttctatgtacgacggtgctctgttcaaaatcctgatgaacaccatcccgtctcacgcgaccgttatcggtatcggtgacgaagaacagctgcgtccggtaagcccgggtgactctctgccgtctaaatctccgttcttctctgactctcgtttcaaacaggttaccctgaccgaagttaaacgttctaacggtccgatcatcaaagttgctaccgaaatccgtaccggtggttggttccgtgaatgcatcgaagacggtcacggtttccacggtttcggtggtgacaaaccgctgcagcagtacatgatgaaatacttcgacgttgttaaatctccggaagacctgttcgaaacccgtatgctggcttacaccaacaaatctgttgacaaactgaacggtatcatccgtcgtaaactgtacgaaaccgaaaacccgttcatcgttggtgaagttctggttatgcaggaaccgtacatgaaacagctggaatttgacggtaaaaaattcaacgaaatcatcttcaacaacggtcagatgatccgtatcctggactgcaaactgacctctaccttcctgaaagctcgtgacgtttctgttaaacagatgatctcttactggcacctggaagttgaaaccgttgacgaagacgacgactaccagcgtgaaaccatcaaagttctggctgacgctaacgaaaaacagaaattcgacatgttcctggctaaagtttgcaccacctaccgtgaactgaaatctgctggtcgtcgtccgcactgggctgacttctgggacgctaaacgtaccttcctgaaagttaaagctctgccgtgctctaccatccacaaatctcagggtatctctgttgacaacaccttcatctacaccccgtgcatcaccctggctgacatcgacctggctaaacagctggcttacgtttctgctacccgtgctcgtcatgacgtgtacttcgtctaa

SEQ ID NO: 34 - DNA, 1332 bp, Artificial Sequence
atgaccatcggtttcgacgacctgaccgaaggtcagaaatgcgctttcgaaaccgctgttgaactggttaactctaaacgtaaacacatgaccctgaacggtccggctggttctggtaaaaccacttggaccaggttcttcatcgaccatctggttcgttctggtgaatctggtgttatcctggctgctccgacccaccaggctaaaaaagttctgtctaaactgtctggtgttgaagcttctaccatccactctatcctgaaaatcaacccgaccacctacgaatgcaacgttctgttcgaacagaaagaaatcccggacctggctaaatgccgtgttctgatctgcgacgaagcttctatgtacgaccgtaaactgttcgacatcctgatgaactctatcccgtcttgggcgatcgttatcgctctgggtgacaaagaccagctgcgtccggttgaactgaactctgaaggtaaaggtcagatctctgctttcttctacgacccgcgtttcgaacaggttttcctgtctgaaatcaaacgttctaactctccgatcatcgaagttgctacctctatccgtaccggtggttggctgtaccacaacctgggtgacgacggtaccggtgttcacggttacatgaacaaaggttctgctctgaaagacttcttcggtcagtacttcgacaccgttcgtaaaccggaagacctgttcgaaaaccgtatgtgcgcttacaccaacgaatctgttaacaaactgaactctatcatccgtcgtaaaatctacgacaccgaagacccgttcgttgttaacgaagttctggttatgcaggaaccgctgaccaaagaaatcaaattcgaaggtaaacgtttctctgaaatgatcttccacaacggtcagatggttcgtgttgttaaagctgaaaaaacctctaaattcctgcgtgctaaaggtgtttctggtgaacagatgatccgttactggtctctggttgttgaaaccaacgacgctgaagacgaatacttccgtgaacagatctgcgttctgtctgacgaaaacgaaatcaacaaatactactacttcctggctaaagtttgcgacgcttacaaatctggtgctgttaaagctcactgggctgacttctgggctgctaaacgtgctttcatcaaagttaaagctctgccgtgctctaccatccacaaagttcagggtatctctgttgacaactgcttcctgtacaccccgtgcatccacaaagctgacgctgacctggctaaacagctgacctacgttggtgctacccgtccgcgtttcaacctgcactacgtttaa

SEQ ID NO: 35 - DNA, 1326 bp, Artificial Sequence
atgatcaccatcgaccagctgaccgaaggtcagttcgactctctgcagcgtgctaaagttctgatccaggaagctaccaaaaacgacggtaactggaaccaccgtaccaaacacctgaccatcaacggtccggctggtaccggtaaaaccaccatgatgaaattcctggtttcttggctgcgtgacgaaggtatcaccggtgttgctctggctgctccgacccacgctgctaaaaaagttctggctaacgctgttggtgaagaagtttctaccatccactctatcctgaaaatcaacccgaccacctacgaatgcaaacagttcttcgaacagtctgctccgccggacctgtctaaaatccgtatcctgatctgcgaagaatgctctttctacgacatcaaactgttcgaaatcctgatgaactctatccagccgtggaccatcatcatcggtatcggtgaccgtgctcagctgcgtccggctgacgacaaaggtatctctcgtttcttcaccgaccagcgtttcgaacagacctacctgaccgaaatcaaacgttctaacatgccgatcatcgaagttgctaccgaaatccgtaacggtggttggattcgtgaaaacatcatcgacgacctgggtgttaaacaggacaaatctgtttctgaatttatgaccaactacttcaaagttgttaaatctatcgacgacctgtacgaaacccgtatgtacgcttacaccaacaactctgttgacaccctgaacaaaatcatccgtaaaaaactgtacgaaaccgaacaggacttcatcgttggtgaaccgatcgttatgcaggaaccgctgatccgtgacatcaactacgaaggtaaacgtttccaggaaatcgttttcaacaacggtgaatacctggaagtttctgaaatcaaaccgatggaatctgttctgaaatgccgtaacatcgactaccagctggttctgcactactaccagctgaaagttaaatctatcgacaccggtgaatctggtctgatcaacaccatctctgacaaaaacgaactgaacaaattctacatgttcctgggtaaagtttgccaggactacaaatctggtaccatcaaagcgttctgggacgacttctggaaaatcaaaaacaactaccaccgtgttaaaccgctgccggtttctaccatccacaaaggtcagggttctaccgttgacaactctttcctgtacaccccgtgcatcaccaaatacgctgaaccggacctggcttctcagctgctgtacgttggtgttacccgtgctcgtcacaacgttaacttcgttggttaa